European Patent Specification EP 3 420 348 B1, published June 7, 2023. Title: METHODS FOR PREVENTING OR REDUCING ACUTE KIDNEY INJURY. Applicant: Mitin, Natalia. The sequence listing filed with the application follows.

SEQUENCE LISTING (32 sequences)

SEQ ID NO: 1 - DNA, 9 bp, Artificial Sequence
  Sequence crosses natural Exon 1-Exon 2 boundary with no intron
ccaggtcat

SEQ ID NO: 2 - DNA, 146 bp, Homo sapiens
atggagccggcggcggggagcagcatggagccttcggctgactggctggccacggccgcggcccggggtcgggtagaggaggtgcgggcgctgctggaggcgggggcgctgcccaacgcaccgaatagttacggtcggaggccgat

SEQ ID NO: 3 - DNA, 189 bp, Homo sapiens
atggtgcgcaggttcttggtgaccctccggattcggcgcgcgtgcggcccgccgcgagtgagggttttcgtggttcacatcccgcggctcacgggggagtgggcagcgccaggggcgcccgccgctgtggccctcgtgctgatgctactgaggagccagcgtctagggcagcagccgcttcctagaaga

SEQ ID NO: 4 - DNA, 201 bp, Homo sapiens
gatgatgggcagcgcccgagtggcggagctgctgctgctccacggcgcggagcccaactgcgccgaccccgccactctcacccgacccgtgcacgacgctgcccgggagggcttcctggacacgctggtggtgctgcaccgggccggggcgcggctggacgtgcgcgatgcctggggccgtctgcccgtggacctggctga

SEQ ID NO: 5 - DNA, 316 bp, Homo sapiens
gatgatgggcagcgcccgagtggcggagctgctgctgctccacggcgcggagcccaactgcgccgaccccgccactctcacccgacccgtgcacgacgctgcccgggagggcttcctggacacgctggtggtgctgcaccgggccggggcgcggctggacgtgcgcgatgcctggggccgtctgcccgtggacctggctgaggagctgggccatcgcgatgtcgcacggtacctgcgcgcggctgcggggggcaccagaggcagtaaccatgcccgcatagatgccgcggaaggtccctcagacatccccgattga

SEQ ID NO: 6 - DNA, 58 bp, Artificial Sequence
  Sequence crosses natural Exon 1-Exon 2 boundary with no intron
ccaacgcaccgaatagttacggtcggaggccgatccaggtcatgatgatgggcagcgc

SEQ ID NO: 7 - DNA, 60 bp, Artificial Sequence
  Sequence crosses natural Exon 1-Exon 2 boundary with no intron
ctgaggagccagcgtctagggcagcagccgcttcctagaagaccaggtcatgatgatggg

SEQ ID NO: 8 - DNA, 21 bp, Artificial Sequence
  Synthetic Primer
ccaacgcaccgaatagttacg

SEQ ID NO: 9 - DNA, 18 bp, Artificial Sequence
  Synthetic Primer
gcgctgcccatcatcatg

SEQ ID NO: 10 - DNA, 18 bp, Artificial Sequence
  Synthetic Probe
  misc_feature (1)..(1): 5' labeled with FAM
  misc_feature (18)..(18): 3' labeled with MGB and NFQ
cctggatcggcctccgac

SEQ ID NO: 11 - DNA, 19 bp, Artificial Sequence
  Synthetic Primer
ctgaggagccagcgtctag

SEQ ID NO: 12 - DNA, 25 bp, Artificial Sequence
  Synthetic Primer
cccatcatcatgacctggtcttcta

SEQ ID NO: 13 - DNA, 14 bp, Artificial Sequence
  Synthetic Probe
  misc_feature (1)..(1): 5' labelled with FAM
  misc_feature (14)..(14): 3' labelled with MGB and NFQ
cagcagccgcttcc

SEQ ID NO: 14 - DNA, 471 bp, Artificial Sequence
  Coding sequence includes Exon boundaries with no intervening intron
atggagccggcggcggggagcagcatggagccttcggctgactggctggccacggccgcggcccggggtcgggtagaggaggtgcgggcgctgctggaggcgggggcgctgcccaacgcaccgaatagttacggtcggaggccgatccaggtcatgatgatgggcagcgcccgagtggcggagctgctgctgctccacggcgcggagcccaactgcgccgaccccgccactctcacccgacccgtgcacgacgctgcccgggagggcttcctggacacgctggtggtgctgcaccgggccggggcgcggctggacgtgcgcgatgcctggggccgtctgcccgtggacctggctgaggagctgggccatcgcgatgtcgcacggtacctgcgcgcggctgcggggggcaccagaggcagtaaccatgcccgcatagatgccgcggaaggtccctcagacatccccgattga

SEQ ID NO: 15 - DNA, 399 bp, Artificial Sequence
  Coding sequence includes Exon boundaries with no intervening intron
atggtgcgcaggttcttggtgaccctccggattcggcgcgcgtgcggcccgccgcgagtgagggttttcgtggttcacatcccgcggctcacgggggagtgggcagcgccaggggcgcccgccgctgtggccctcgtgctgatgctactgaggagccagcgtctagggcagcagccgcttcctagaagaccaggtcatgatgatgggcagcgcccgagtggcggagctgctgctgctccacggcgcggagcccaactgcgccgaccccgccactctcacccgacccgtgcacgacgctgcccgggagggcttcctggacacgctggtggtgctgcaccgggccggggcgcggctggacgtgcgcgatgcctggggccgtctgcccgtggacctggctga

SEQ ID NO: 16 - DNA, 19 bp, Artificial Sequence
  Synthetic Primer
ctcgtgctgatgctactga

SEQ ID NO: 17 - DNA, 20 bp, Artificial Sequence
  Synthetic Primer
tcatcatgacctggtcttct

SEQ ID NO: 18 - DNA, 20 bp, Artificial Sequence
  Synthetic Probe
  misc_feature (1)..(1): 5' modified with FAM
  misc_feature (20)..(20): 3' modified with BHQ1a-Q
aagcggctgctgccctagac

SEQ ID NO: 19 - DNA, 306 bp, Homo sapiens
cgagggctgcttccggctggtgcccccgggggagacccaacctggggcgacttcaggggtgccacattcgctaagtgctcggagttaatagcacctcctccgagcactcgctcacggcgtccccttgcctggaaagataccgcggtccctccagaggatttgagggacagggtcggagggggctcttccgccagcaccggaggaagaaagaggaggggctggctggtcaccagagggtggggcggaccgcgtgcgctcggcggctgcggagagggggagagcaggcagcgggcggcggggagcagc

SEQ ID NO: 20 - DNA, 490 bp, Homo sapiens
aagaaccagagaggctctgagaaacctcgggaaacttagatcatcagtcaccgaaggtcctacagggccacaactgcccccgccacaacccaccccgctttcgtagttttcatttagaaaatagagcttttaaaaatgtcctgccttttaacgtagatatatgccttcccccactaccgtaaatgtccatttatatcattttttatatattcttataaaaatgtaaaaaagaaaaacaccgcttctgccttttcactgtgttggagttttctggagtgagcactcacgccctaagcgcacattcatgtgggcatttcttgcgagcctcgcagcctccggaagctgtcgacttcatgacaagcattttgtgaactagggaagctcaggggggttactggcttctcttgagtcacactgctagcaaatggcagaaccaaagctcaaataaaaataaaataattttcattcattcactcaaaaaaaaaaaaaa

SEQ ID NO: 21 - DNA, 160 bp, Homo sapiens
cgctcagggaaggcgggtgcgcgcctgcggggcggagatgggcagggggcggtgcgtgggtcccagtctgcagttaagggggcaggagtggcgctgctcacctctggtgccaaagggcggcgcagcggctgccgagctcggccctggaggcggcgagaac

SEQ ID NO: 22 - DNA, 605 bp, Homo sapiens
ggagctgggccatcgcgatgtcgcacggtacctgcgcgcggctgcggggggcaccagaggcagtaaccatgcccgcatagatgccgcggaaggtccctcagacatccccgattgaaagaaccagagaggctctgagaaacctcgggaaacttagatcatcagtcaccgaaggtcctacagggccacaactgcccccgccacaacccaccccgctttcgtagttttcatttagaaaatagagcttttaaaaatgtcctgccttttaacgtagatatatgccttcccccactaccgtaaatgtccatttatatcattttttatatattcttataaaaatgtaaaaaagaaaaacaccgcttctgccttttcactgtgttggagttttctggagtgagcactcacgccctaagcgcacattcatgtgggcatttcttgcgagcctcgcagcctccggaagctgtcgacttcatgacaagcattttgtgaactagggaagctcaggggggttactggcttctcttgagtcacactgctagcaaatggcagaaccaaagctcaaataaaaataaaataattttcattcattcactcaaaaaaaaaaaaaa

SEQ ID NO: 23 - DNA, 1267 bp, Homo sapiens
cgagggctgcttccggctggtgcccccgggggagacccaacctggggcgacttcaggggtgccacattcgctaagtgctcggagttaatagcacctcctccgagcactcgctcacggcgtccccttgcctggaaagataccgcggtccctccagaggatttgagggacagggtcggagggggctcttccgccagcaccggaggaagaaagaggaggggctggctggtcaccagagggtggggcggaccgcgtgcgctcggcggctgcggagagggggagagcaggcagcgggcggcggggagcagcatggagccggcggcggggagcagcatggagccttcggctgactggctggccacggccgcggcccggggtcgggtagaggaggtgcgggcgctgctggaggcgggggcgctgcccaacgcaccgaatagttacggtcggaggccgatccaggtcatgatgatgggcagcgcccgagtggcggagctgctgctgctccacggcgcggagcccaactgcgccgaccccgccactctcacccgacccgtgcacgacgctgcccgggagggcttcctggacacgctggtggtgctgcaccgggccggggcgcggctggacgtgcgcgatgcctggggccgtctgcccgtggacctggctgaggagctgggccatcgcgatgtcgcacggtacctgcgcgcggctgcggggggcaccagaggcagtaaccatgcccgcatagatgccgcggaaggtccctcagacatccccgattgaaagaaccagagaggctctgagaaacctcgggaaacttagatcatcagtcaccgaaggtcctacagggccacaactgcccccgccacaacccaccccgctttcgtagttttcatttagaaaatagagcttttaaaaatgtcctgccttttaacgtagatatatgccttcccccactaccgtaaatgtccatttatatcattttttatatattcttataaaaatgtaaaaaagaaaaacaccgcttctgccttttcactgtgttggagttttctggagtgagcactcacgccctaagcgcacattcatgtgggcatttcttgcgagcctcgcagcctccggaagctgtcgacttcatgacaagcattttgtgaactagggaagctcaggggggttactggcttctcttgagtcacactgctagcaaatggcagaaccaaagctcaaataaaaataaaataattttcattcattcactcaaaaaaaaaaaaaa

SEQ ID NO: 24 - DNA, 1164 bp, Homo sapiens
cgctcagggaaggcgggtgcgcgcctgcggggcggagatgggcagggggcggtgcgtgggtcccagtctgcagttaagggggcaggagtggcgctgctcacctctggtgccaaagggcggcgcagcggctgccgagctcggccctggaggcggcgagaacatggtgcgcaggttcttggtgaccctccggattcggcgcgcgtgcggcccgccgcgagtgagggttttcgtggttcacatcccgcggctcacgggggagtgggcagcgccaggggcgcccgccgctgtggccctcgtgctgatgctactgaggagccagcgtctagggcagcagccgcttcctagaagaccaggtcatgatgatgggcagcgcccgagtggcggagctgctgctgctccacggcgcggagcccaactgcgccgaccccgccactctcacccgacccgtgcacgacgctgcccgggagggcttcctggacacgctggtggtgctgcaccgggccggggcgcggctggacgtgcgcgatgcctggggccgtctgcccgtggacctggctgaggagctgggccatcgcgatgtcgcacggtacctgcgcgcggctgcggggggcaccagaggcagtaaccatgcccgcatagatgccgcggaaggtccctcagacatccccgattgaaagaaccagagaggctctgagaaacctcgggaaacttagatcatcagtcaccgaaggtcctacagggccacaactgcccccgccacaacccaccccgctttcgtagttttcatttagaaaatagagcttttaaaaatgtcctgccttttaacgtagatatatgccttcccccactaccgtaaatgtccatttatatcattttttatatattcttataaaaatgtaaaaaagaaaaacaccgcttctgccttttcactgtgttggagttttctggagtgagcactcacgccctaagcgcacattcatgtgggcatttcttgcgagcctcgcagcctccggaagctgtcgacttcatgacaagcattttgtgaactagggaagctcaggggggttactggcttctcttgagtcacactgctagcaaatggcagaaccaaagctcaaataaaaataaaataattttcattcattcactcaaaaaaaaaaaaaa

SEQ ID NO: 25 - DNA, 71 bp, Artificial Sequence
  Synthetic Sequence
ctcgtgctgatgctactgaggagccagcgtctagggcagcagccgcttcctagaagaccaggtcatgatga

SEQ ID NO: 26 - DNA, 20 bp, Artificial Sequence
  Synthetic Primer
tgatgacaagaaagggattg

SEQ ID NO: 27 - DNA, 21 bp, Artificial Sequence
  Synthetic Primer
cccagtctgataggatgtgtt

SEQ ID NO: 28 - DNA, 25 bp, Artificial Sequence
  Synthetic Probe
  misc_feature (1)..(1): 5' labeled with FAM
  misc_feature (25)..(25): 3' labeled with 3BHQ_1
tcgatcagtcacaacaagcatacca

SEQ ID NO: 29 - DNA, 353 bp, Homo sapiens
cgctcagggaaggcgggtgcgcgcctgcggggcggagatgggcagggggcggtgcgtgggtcccagtctgcagttaagggggcaggagtggcgctgctcacctctggtgccaaagggcggcgcagcggctgccgagctcggccctggaggcggcgagaacatggtgcgcaggttcttggtgaccctccggattcggcgcgcgtgcggcccgccgcgagtgagggttttcgtggttcacatcccgcggctcacgggggagtgggcagcgccaggggcgcccgccgctgtggccctcgtgctgatgctactgaggagccagcgtctagggcagcagccgcttcctagaagaccag

SEQ ID NO: 30 - DNA, 456 bp, Homo sapiens
cgagggctgcttccggctggtgcccccgggggagacccaacctggggcgacttcaggggtgccacattcgctaagtgctcggagttaatagcacctcctccgagcactcgctcacggcgtccccttgcctggaaagataccgcggtccctccagaggatttgagggacagggtcggagggggctcttccgccagcaccggaggaagaaagaggaggggctggctggtcaccagagggtggggcggaccgcgtgcgctcggcggctgcggagagggggagagcaggcagcgggcggcggggagcagcatggagccggcggcggggagcagcatggagccttcggctgactggctggccacggccgcggcccggggtcgggtagaggaggtgcgggcgctgctggaggcgggggcgctgcccaacgcaccgaatagttacggtcggaggccgatccag

SEQ ID NO: 31 - DNA, 307 bp, Homo sapiens
gtcatgatgatgggcagcgcccgagtggcggagctgctgctgctccacggcgcggagcccaactgcgccgaccccgccactctcacccgacccgtgcacgacgctgcccgggagggcttcctggacacgctggtggtgctgcaccgggccggggcgcggctggacgtgcgcgatgcctggggccgtctgcccgtggacctggctgaggagctgggccatcgcgatgtcgcacggtacctgcgcgcggctgcggggggcaccagaggcagtaaccatgcccgcatagatgccgcggaaggtccctcag

SEQ ID NO: 32 - DNA, 504 bp, Homo sapiens
acatccccgattgaaagaaccagagaggctctgagaaacctcgggaaacttagatcatcagtcaccgaaggtcctacagggccacaactgcccccgccacaacccaccccgctttcgtagttttcatttagaaaatagagcttttaaaaatgtcctgccttttaacgtagatatatgccttcccccactaccgtaaatgtccatttatatcattttttatatattcttataaaaatgtaaaaaagaaaaacaccgcttctgccttttcactgtgttggagttttctggagtgagcactcacgccctaagcgcacattcatgtgggcatttcttgcgagcctcgcagcctccggaagctgtcgacttcatgacaagcattttgtgaactagggaagctcaggggggttactggcttctcttgagtcacactgctagcaaatggcagaaccaaagctcaaataaaaataaaataattttcattcattcactcaaaaaaaaaaaaaa